European Patent Application EP 4 148 133 A1, published March 15, 2023. Title: Chimeric protein containing fibrinogen fragment and laminin fragment and use thereof. Applicant: Osaka University MATRIXOME, Inc. The sequence listing filed with the application follows.

SEQUENCE LISTING (40 sequences)

SEQ ID NO: 1 - DNA, 50 bp, Artificial Sequence
  Primer
gggagacccaagctggctagccaccatgttttccatgaggatcgtctgcc

SEQ ID NO: 2 - DNA, 37 bp, Artificial Sequence
  Primer
tcctcgagcggccgccgatctagggggacagggaagg

SEQ ID NO: 3 - DNA, 55 bp, Artificial Sequence
  Primer
tagggagacccaagctggctagccaccatgaaaaggatggtttcttggagcttcc

SEQ ID NO: 4 - DNA, 40 bp, Artificial Sequence
  Primer
cctcctcgagcggccgcgatctattgctgtgggaagaagg

SEQ ID NO: 5 - DNA, 43 bp, Artificial Sequence
  Primer
acccaagctggctagccaccatgagttggtccttgcacccccg

SEQ ID NO: 6 - DNA, 44 bp, Artificial Sequence
  Primer
ccctcctcgagcggccgcgatttaaacgtctccagcctgtttgg

SEQ ID NO: 7 - DNA, 34 bp, Artificial Sequence
  Primer
agcctgcgatggctcttccccaccggaggctcag

SEQ ID NO: 8 - DNA, 41 bp, Artificial Sequence
  Primer
gtgatggtgatggtgatggtgatggtgatgggcctgcagtc

SEQ ID NO: 9 - DNA, 47 bp, Artificial Sequence
  Primer
aggcccatcaccatcaccatcaccatcaccatcactagatccagcac

SEQ ID NO: 10 - DNA, 46 bp, Artificial Sequence
  Primer
gatcgaacccttgatggctggcaactagaaggcacagtcgaggctg

SEQ ID NO: 11 - DNA, 37 bp, Artificial Sequence
  Primer
agctcgtttagtgaaccgtcagatcgcctggagacgc

SEQ ID NO: 12 - DNA, 57 bp, Artificial Sequence
  Primer
gaacggacttctccttccagtcttgctaaatgctgtactttttctatgactttgcgc

SEQ ID NO: 13 - DNA, 41 bp, Artificial Sequence
  Primer
gctctcgcacgcggccaatgttagttgggatattgctattc

SEQ ID NO: 14 - DNA, 53 bp, Artificial Sequence
  Primer
gcgaatgtccttcatgatctcctcgatacttgagtcatgtgttaaaatcgatg

SEQ ID NO: 15 - DNA, 41 bp, Artificial Sequence
  Primer
gaatagcaatatcccaactaacattggccgcgtgcgagagc

SEQ ID NO: 16 - DNA, 36 bp, Artificial Sequence
  Primer
ccttgatggctggcaactagaaggcacagtcgaggc

SEQ ID NO: 17 - DNA, 57 bp, Artificial Sequence
  Primer
gcgcaaagtcatagaaaaagtacagcatttagcaagactggaaggagaagtccgttc

SEQ ID NO: 18 - DNA, 53 bp, Artificial Sequence
  Primer
catcgattttaacacatgactcaagtatcgaggagatcatgaaggacattcgc

SEQ ID NO: 19 - DNA, 49 bp, Artificial Sequence
  Primer
ctatataagcagagctcgtttagtgaaccgtcagatcgcctggagacgc

SEQ ID NO: 20 - DNA, 37 bp, Artificial Sequence
  Primer
cattgtcgttgacaccttggtcaccagtggaacctgg

SEQ ID NO: 21 - DNA, 38 bp, Artificial Sequence
  Primer
caccttcaccactatctgcgtcaccagtggaacctgga

SEQ ID NO: 22 - DNA, 46 bp, Artificial Sequence
  Primer
cagttgtctctggtagcaacatagtcaccagtggaacctggaaccc

SEQ ID NO: 23 - DNA, 37 bp, Artificial Sequence
  Primer
ccaggttccactggtgaccaaggtgtcaacgacaatg

SEQ ID NO: 24 - DNA, 39 bp, Artificial Sequence
  Primer
ccggtagggatcgaacccttgatggctggcaactagaag

SEQ ID NO: 25 - DNA, 38 bp, Artificial Sequence
  Primer
tccaggttccactggtgacgcagatagtggtgaaggtg

SEQ ID NO: 26 - DNA, 46 bp, Artificial Sequence
  Primer
gggttccaggttccactggtgactatgttgctaccagagacaactg

SEQ ID NO: 27 - DNA, 41 bp, Artificial Sequence
  Primer
cgggactttccaaaatgtcgtaacaactccgccccattgac

SEQ ID NO: 28 - DNA, 50 bp, Artificial Sequence
  Primer
caatgagctctcgcacgcggccaatatgctgtactttttctatgactttg

SEQ ID NO: 29 - DNA, 50 bp, Artificial Sequence
  Primer
caaagtcatagaaaaagtacagcatattggccgcgtgcgagagctcattg

SEQ ID NO: 30 - DNA, 37 bp, Artificial Sequence
  Primer
cccttgatggctggcaactagaaggcacagtcgaggc

SEQ ID NO: 31 - DNA, 60 bp, Artificial Sequence
  Primer
gagtgaacggacttctccttccagtcttgctaaacttgagtcatgtgttaaaatcgatgc

SEQ ID NO: 32 - DNA, 60 bp, Artificial Sequence
  Primer
gcatcgattttaacacatgactcaagtttagcaagactggaaggagaagtccgttcactc

SEQ ID NO: 33 - DNA, 60 bp, Artificial Sequence
  Primer
gcgaatgtccttcatgatctcctcgatgttagttgggatattgctattcacagtctcatc

SEQ ID NO: 34 - DNA, 60 bp, Artificial Sequence
  Primer
gatgagactgtgaatagcaatatcccaactaacatcgaggagatcatgaaggacattcgc

SEQ ID NO: 35 - DNA, 44 bp, Artificial Sequence
  Primer
gagctctcgcacgcggccaatacttgagtcatgtgttaaaatcg

SEQ ID NO: 36 - DNA, 44 bp, Artificial Sequence
  Primer
cgattttaacacatgactcaagtattggccgcgtgcgagagctc

SEQ ID NO: 37 - DNA, 67 bp, Artificial Sequence
  Primer
ggagtgaacggacttctccttccagtcttgctaagttagttgggatattgctattcacagtctcatc

SEQ ID NO: 38 - DNA, 67 bp, Artificial Sequence
  Primer
gatgagactgtgaatagcaatatcccaactaacttagcaagactggaaggagaagtccgttcactcc

SEQ ID NO: 39 - DNA, 58 bp, Artificial Sequence
  Primer
gcgaatgtccttcatgatctcctcgatatgctgtactttttctatgactttgcgcttc

SEQ ID NO: 40 - DNA, 58 bp, Artificial Sequence
  Primer
gaagcgcaaagtcatagaaaaagtacagcatatcgaggagatcatgaaggacattcgc